European Patent Application EP 4 582 451 A1, published July 9, 2025. Title: ANTIBODY BINDING TO THYROID-STIMULATING HORMONE RECEPTOR AND USE THEREOF. Applicant: CHANGCHUN GENESCIENCE PHARMACEUTICAL CO., LTD. Application CN. The sequence listing filed with the application follows.

SEQUENCE LISTING (55 sequences)

SEQ ID NO: 1 - protein, 119 aa, synthetic construct
  source 1..119: note = mAb001 VH
EVQLVESGGGLVKPGGSLKLSCAASGFTLSDYYIYWVRQTPEKRLEWVATISDGVIYTYYADSVKGRFTISRDNAKNNLYLQMSSLKSEDTAMYFCARAYGSSEVMDYWGQGTSVTVSS

SEQ ID NO: 2 - protein, 10 aa, synthetic construct
  source 1..10: note = mAb001 VH CDR1
GFTLSDYYIY

SEQ ID NO: 3 - protein, 17 aa, synthetic construct
  source 1..17: note = mAb001 VH CDR2
TISDGVIYTYYADSVKG

SEQ ID NO: 4 - protein, 10 aa, synthetic construct
  source 1..10: note = mAb001 VH CDR3
AYGSSEVMDY

SEQ ID NO: 5 - protein, 106 aa, synthetic construct
  source 1..106: note = mAb001 VL
QIVLTQSPAVLSASPGEKVTMTCSASSSVSYMHWYQQKSGTSPKRWIYDTSKLASGVPARFSGSGSGTSYSLTISSMEAEDAATYYCQQWSSNPWTFGGGTKLEIK

SEQ ID NO: 6 - protein, 10 aa, synthetic construct
  source 1..10: note = mAb001 VL CDR1
SASSSVSYMH

SEQ ID NO: 7 - protein, 7 aa, synthetic construct
  source 1..7: note = mAb001 VL CDR2
DTSKLAS

SEQ ID NO: 8 - protein, 9 aa, synthetic construct
  source 1..9: note = mAb001 VL CDR3
QQWSSNPWT

SEQ ID NO: 9 - protein, 119 aa, synthetic construct
  source 1..119: note = mAb012 VH
EVQLQQSGPVLLKPGASVKMSCKASGYTFTDYYMNWVKQSHGKSLEWIGVINPYNGESSNNQKFKGKATMTVDKSSSTAYMELNSLTSEDSAVYYCARCYGYGYYFDYWGQGTTLSVAS

SEQ ID NO: 10 - protein, 10 aa, synthetic construct
  source 1..10: note = mAb012 VH CDR1
GYTFTDYYMN

SEQ ID NO: 11 - protein, 17 aa, synthetic construct
  source 1..17: note = mAb012 VH CDR2
VINPYNGESSNNQKFKG

SEQ ID NO: 12 - protein, 10 aa, synthetic construct
  source 1..10: note = mAb012 VH CDR3
CYGYGYYFDY

SEQ ID NO: 13 - protein, 106 aa, synthetic construct
  source 1..106: note = mAb012 VL
QIVLTQSPAIMSASPGEKVTMTCSATSSVTYMHWYQQKSGTSPKRWIYDTSKLTSGVPPRFSGSGSGTSYSLTISSMEAEDAATYYCQQWSTYPYTFGGGTKLEIK

SEQ ID NO: 14 - protein, 10 aa, synthetic construct
  source 1..10: note = mAb012 VL CDR1
SATSSVTYMH

SEQ ID NO: 15 - protein, 7 aa, synthetic construct
  source 1..7: note = mAb012 VL CDR2
DTSKLTS

SEQ ID NO: 16 - protein, 9 aa, synthetic construct
  source 1..9: note = mAb012 VL CDR3
QQWSTYPYT

SEQ ID NO: 17 - protein, 118 aa, synthetic construct
  source 1..118: note = mAb021 VH
QVQLQQPGAEHVQPGASVKLSCKASGYTFSNYWMQWVRQRPGQGLDWIGEIDPADSYTAYSQKFKGKATLTVDTSSTTAYMQLSSLTSEDSAVYYCARRNLLRSGDYWGQGTSLTVSS

SEQ ID NO: 18 - protein, 10 aa, synthetic construct
  source 1..10: note = mAb021 VH CDR1
GYTFSNYWMQ

SEQ ID NO: 19 - protein, 17 aa, synthetic construct
  source 1..17: note = mAb021 VH CDR2
EIDPADSYTAYSQKFKG

SEQ ID NO: 20 - protein, 9 aa, synthetic construct
  source 1..9: note = mAb021 VH CDR3
RNLLRSGDY

SEQ ID NO: 21 - protein, 106 aa, synthetic construct
  source 1..106: note = mAb021 VL
QIVLTQSPAIMSASPGEKVTMTCSASSGITYIHWYQQKSGTSPKRWIYDSSKLASGVPARFSGSGSGTSYSLTISSMEAEDAATYYCQQWSGNPPTFGAGTKLEVK

SEQ ID NO: 22 - protein, 10 aa, synthetic construct
  source 1..10: note = mAb021 VL CDR1
SASSGITYIH

SEQ ID NO: 23 - protein, 7 aa, synthetic construct
  source 1..7: note = mAb021 VL CDR2
DSSKLAS

SEQ ID NO: 24 - protein, 9 aa, synthetic construct
  source 1..9: note = mAb021 VL CDR3
QQWSGNPPT

SEQ ID NO: 25 - protein, 327 aa, synthetic construct
  source 1..327: note = the constant region of human IgG4-S228P heavy chain
ASTKGPSVFPLAPCSRSTSESTAALGCLVKDYFPEPVTVSWNSGALTSGVHTFPAVLQSSGLYSLSSVVTVPSSSLGTKTYTCNVDHKPSNTKVDKRVESKYGPPCPPCPAPEFLGGPSVFLFPPKPKDTLMISRTPEVTCVVVDVSQEDPEVQFNWYVDGVEVHNAKTKPREEQFNSTYRVVSVLTVLHQDWLNGKEYKCKVSNKGLPSSIEKTISKAKGQPREPQVYTLPPSQEEMTKNQVSLTCLVKGFYPSDIAVEWESNGQPENNYKTTPPVLDSDGSFFLYSRLTVDKSRWQEGNVFSCSVMHEALHNHYTQKSLSLSLGK

SEQ ID NO: 26 - protein, 107 aa, synthetic construct [sequence omitted]

SEQ ID NO: 27 - protein, 119 aa, synthetic construct
  source 1..119: note = VH of cAb01-VH1-DA-VL2/cAb01-VH1-DA-VL3
EVQLVESGGGLVKPGGSLRLSCAASGFTLSDYYIYWVRQAPGKGLEWVSTISDAVIYTYYADSVKGRFTISRDNAKNSLYLQMNSLRAEDTAVYYCARAYGSSEVMDYWGQGTLVTVSS

SEQ ID NO: 28 - protein, 106 aa, synthetic construct
  source 1..106: note = VL of cAb01-VH1-DA-VL2/cAb01-VH2-DA-VL2/cAb01-VH3-DA-VL2
EIVLTQSPATLSLSPGERATLSCSASSSVSYMHWYQQKPGQAPRRWIYDTSKLASGIPARFSGSGSGTDYTLTISSLEPEDFAVYYCQQWSSNPWTFGGGTKLEIK

SEQ ID NO: 29 - protein, 119 aa, synthetic construct
  source 1..119: note = VH of cAb01-VH2-DA-VL2/cAb01-VH2-DA-VL3
EVQLVESGGGLVKPGGSLRLSCAASGFTLSDYYIYWVRQAPGKGLEWVATISDAVIYTYYADSVKGRFTISRDNAKNSLYLQMNSLRAEDTAVYFCARAYGSSEVMDYWGQGTLVTVSS

SEQ ID NO: 30 - protein, 119 aa, synthetic construct
  source 1..119: note = VH of cAb01-VH3-DA-VL2
EVQLVESGGGLVKPGGSLRLSCAASGFTLSDYYIYWVRQAPGKRLEWVATISDAVIYTYYADSVKGRFTISRDNAKNSLYLQMNSLRAEDTAVYFCARAYGSSEVMDYWGQGTLVTVSS

SEQ ID NO: 31 - protein, 106 aa, synthetic construct
  source 1..106: note = VL of cAb01-VH1-DA-VL3/cAb01-VH2-DA-VL3
EIVLTQSPATLSLSPGERATLSCSASSSVSYMHWYQQKPGQAPKRWIYDTSKLASGVPARFSGSGSGTDYTLTISSLEPEDFAVYYCQQWSSNPWTFGGGTKLEIK

SEQ ID NO: 32 - protein, 119 aa, synthetic construct
  source 1..119: note = VH of cAb12-VH1-QG&S-VL3
QVQLVQSGAEVKKPGASVKVSCKASGYTFTDYYMNWVRQAPGQGLEWMGVINPYQGESSNNQKFKGRVTMTRDTSTSTVYMELSSLRSEDTAVYYCARSYGYGYYFDYWGQGTTVTVSS

SEQ ID NO: 33 - protein, 106 aa, synthetic construct
  source 1..106: note = VL of cAb12-VH1-QG&S-VL3/cAb12-VH3-QG&S-VL3
AIQLTQSPSSLSASVGDRVTITCSATSSVTYMHWYQQKPGKAPKRWIYDTSKLTSGVPPRFSGSGSGTDYTLTISSLQPEDFATYYCQQWSTYPYTFGGGTKLEIK

SEQ ID NO: 34 - protein, 119 aa, synthetic construct
  source 1..119: note = VH of cAb12-VH3-QG&S-VL3
QVQLVQSGAEVKKPGASVKVSCKASGYTFTDYYMNWVKQAPGQGLEWIGVINPYQGESSNNQKFKGRATMTVDKSTSTVYMELSSLRSEDTAVYYCARSYGYGYYFDYWGQGTTVTVSS

SEQ ID NO: 35 - protein, 118 aa, synthetic construct
  source 1..118: note = VH of cAb21-VH2-VL2
QVQLVQSGAEVKKPGASVKVSCKASGYTFSNYWMQWVRQAPGQGLEWIGEIDPADSYTAYSQKFKGRATMTVDTSTSTVYMELSSLRSEDTAVYYCARRNLLRSGDYWGQGTLVTVSS

SEQ ID NO: 36 - protein, 106 aa, synthetic construct
  source 1..106: note = VL of cAb21-VH2-VL2
AIQLTQSPSSLSASVGDRVTITCSASSGITYIHWYQQKPGKAPKRWIYDSSKLASGVPSRFSGSGSGTDYTLTISSLQPEDFATYYCQQWSGNPPTFGQGTKLEIK

SEQ ID NO: 37 - protein, 118 aa, synthetic construct
  source 1..118: note = VH of cAb21-VH1-VL3
QVQLVQSGAEVKKPGASVKVSCKASGYTFSNYWMQWVRQAPGQGLEWMGEIDPADSYTAYSQKFKGRVTMTRDTSTSTVYMELSSLRSEDTAVYYCARRNLLRSGDYWGQGTLVTVSS

SEQ ID NO: 38 - protein, 106 aa, synthetic construct
  source 1..106: note = VL of cAb21-VH1-VL3
AIQLTQSPSSLSASVGDRVTITCSASSGITYIHWYQQKPGKAPKRWIYDSSKLASGVPARFSGSGSGTDYTLTISSLQPEDFATYYCQQWSGNPPTFGQGTKLEIK

SEQ ID NO: 39 - protein, 17 aa, synthetic construct
  source 1..17: note = VH CDR2 of cAb01-VH1-DA-VL2/cAb01-VH2-DA-VL2/cAb01-VH3-DA-VL2
TISDAVIYTYYADSVKG

SEQ ID NO: 40 - protein, 17 aa, synthetic construct
  source 1..17: note = VH CDR2 of cAb12-VH1-QG&S-VL3/cAb12-VH3-QG&S-VL3
VINPYQGESSNNQKFKG

SEQ ID NO: 41 - protein, 10 aa, synthetic construct
  source 1..10: note = VH CDR3 of cAb12-VH1-QG&S-VL3/cAb12-VH3-QG&S-VL3
SYGYGYYFDY

SEQ ID NO: 42 - protein, 327 aa, synthetic construct
  source 1..327: note = the constant region of human IgG4-S228P/M252Y/S254T/T256E heavy chain
ASTKGPSVFPLAPCSRSTSESTAALGCLVKDYFPEPVTVSWNSGALTSGVHTFPAVLQSSGLYSLSSVVTVPSSSLGTKTYTCNVDHKPSNTKVDKRVESKYGPPCPPCPAPEFLGGPSVFLFPPKPKDTLYITREPEVTCVVVDVSQEDPEVQFNWYVDGVEVHNAKTKPREEQFNSTYRVVSVLTVLHQDWLNGKEYKCKVSNKGLPSSIEKTISKAKGQPREPQVYTLPPSQEEMTKNQVSLTCLVKGFYPSDIAVEWESNGQPENNYKTTPPVLDSDGSFFLYSRLTVDKSRWQEGNVFSCSVMHEALHNHYTQKSLSLSLGK

SEQ ID NO: 43 - protein, 327 aa, synthetic construct
  source 1..327: note = the constant region of human IgG4-S228P/L235E/M252Y/S254T/T256E heavy chain
ASTKGPSVFPLAPCSRSTSESTAALGCLVKDYFPEPVTVSWNSGALTSGVHTFPAVLQSSGLYSLSSVVTVPSSSLGTKTYTCNVDHKPSNTKVDKRVESKYGPPCPPCPAPEFEGGPSVFLFPPKPKDTLYITREPEVTCVVVDVSQEDPEVQFNWYVDGVEVHNAKTKPREEQFNSTYRVVSVLTVLHQDWLNGKEYKCKVSNKGLPSSIEKTISKAKGQPREPQVYTLPPSQEEMTKNQVSLTCLVKGFYPSDIAVEWESNGQPENNYKTTPPVLDSDGSFFLYSRLTVDKSRWQEGNVFSCSVMHEALHNHYTQKSLSLSLGK

SEQ ID NO: 44 - protein, 330 aa, synthetic construct [sequence omitted]

SEQ ID NO: 45 - protein, 330 aa, synthetic construct
  source 1..330: note = the constant region of human IgG1-L234A/L235A/M252Y/S254T/T256E heavy chain
ASTKGPSVFPLAPSSKSTSGGTAALGCLVKDYFPEPVTVSWNSGALTSGVHTFPAVLQSSGLYSLSSVVTVPSSSLGTQTYICNVNHKPSNTKVDKKVEPKSCDKTHTCPPCPAPEAAGGPSVFLFPPKPKDTLYITREPEVTCVVVDVSHEDPEVKFNWYVDGVEVHNAKTKPREEQYNSTYRVVSVLTVLHQDWLNGKEYKCKVSNKALPAPIEKTISKAKGQPREPQVYTLPPSRDELTKNQVSLTCLVKGFYPSDIAVEWESNGQPENNYKTTPPVLDSDGSFFLYSKLTVDKSRWQQGNVFSCSVMHEALHNHYTQKSLSLSPGK

SEQ ID NO: 46 - protein, 446 aa, synthetic construct
  source 1..446: note = heavy chain of hAb01_G4P
EVQLVESGGGLVKPGGSLRLSCAASGFTLSDYYIYWVRQAPGKGLEWVATISDAVIYTYYADSVKGRFTISRDNAKNSLYLQMNSLRAEDTAVYFCARAYGSSEVMDYWGQGTLVTVSSASTKGPSVFPLAPCSRSTSESTAALGCLVKDYFPEPVTVSWNSGALTSGVHTFPAVLQSSGLYSLSSVVTVPSSSLGTKTYTCNVDHKPSNTKVDKRVESKYGPPCPPCPAPEFLGGPSVFLFPPKPKDTLMISRTPEVTCVVVDVSQEDPEVQFNWYVDGVEVHNAKTKPREEQFNSTYRVVSVLTVLHQDWLNGKEYKCKVSNKGLPSSIEKTISKAKGQPREPQVYTLPPSQEEMTKNQVSLTCLVKGFYPSDIAVEWESNGQPENNYKTTPPVLDSDGSFFLYSRLTVDKSRWQEGNVFSCSVMHEALHNHYTQKSLSLSLGK

SEQ ID NO: 47 - protein, 446 aa, synthetic construct
  source 1..446: note = heavy chain of hAb01_G4P_V1
EVQLVESGGGLVKPGGSLRLSCAASGFTLSDYYIYWVRQAPGKGLEWVATISDAVIYTYYADSVKGRFTISRDNAKNSLYLQMNSLRAEDTAVYFCARAYGSSEVMDYWGQGTLVTVSSASTKGPSVFPLAPCSRSTSESTAALGCLVKDYFPEPVTVSWNSGALTSGVHTFPAVLQSSGLYSLSSVVTVPSSSLGTKTYTCNVDHKPSNTKVDKRVESKYGPPCPPCPAPEFLGGPSVFLFPPKPKDTLYITREPEVTCVVVDVSQEDPEVQFNWYVDGVEVHNAKTKPREEQFNSTYRVVSVLTVLHQDWLNGKEYKCKVSNKGLPSSIEKTISKAKGQPREPQVYTLPPSQEEMTKNQVSLTCLVKGFYPSDIAVEWESNGQPENNYKTTPPVLDSDGSFFLYSRLTVDKSRWQEGNVFSCSVMHEALHNHYTQKSLSLSLGK

SEQ ID NO: 48 - protein, 446 aa, synthetic construct
  source 1..446: note = heavy chain of hAb01_G4P_V2
EVQLVESGGGLVKPGGSLRLSCAASGFTLSDYYIYWVRQAPGKGLEWVATISDAVIYTYYADSVKGRFTISRDNAKNSLYLQMNSLRAEDTAVYFCARAYGSSEVMDYWGQGTLVTVSSASTKGPSVFPLAPCSRSTSESTAALGCLVKDYFPEPVTVSWNSGALTSGVHTFPAVLQSSGLYSLSSVVTVPSSSLGTKTYTCNVDHKPSNTKVDKRVESKYGPPCPPCPAPEFEGGPSVFLFPPKPKDTLYITREPEVTCVVVDVSQEDPEVQFNWYVDGVEVHNAKTKPREEQFNSTYRVVSVLTVLHQDWLNGKEYKCKVSNKGLPSSIEKTISKAKGQPREPQVYTLPPSQEEMTKNQVSLTCLVKGFYPSDIAVEWESNGQPENNYKTTPPVLDSDGSFFLYSRLTVDKSRWQEGNVFSCSVMHEALHNHYTQKSLSLSLGK

SEQ ID NO: 49 - protein, 449 aa, synthetic construct
  source 1..449: note = heavy chain of hAb01_G1
EVQLVESGGGLVKPGGSLRLSCAASGFTLSDYYIYWVRQAPGKGLEWVATISDAVIYTYYADSVKGRFTISRDNAKNSLYLQMNSLRAEDTAVYFCARAYGSSEVMDYWGQGTLVTVSSASTKGPSVFPLAPSSKSTSGGTAALGCLVKDYFPEPVTVSWNSGALTSGVHTFPAVLQSSGLYSLSSVVTVPSSSLGTQTYICNVNHKPSNTKVDKKVEPKSCDKTHTCPPCPAPELLGGPSVFLFPPKPKDTLMISRTPEVTCVVVDVSHEDPEVKFNWYVDGVEVHNAKTKPREEQYNSTYRVVSVLTVLHQDWLNGKEYKCKVSNKALPAPIEKTISKAKGQPREPQVYTLPPSRDELTKNQVSLTCLVKGFYPSDIAVEWESNGQPENNYKTTPPVLDSDGSFFLYSKLTVDKSRWQQGNVFSCSVMHEALHNHYTQKSLSLSPGK

SEQ ID NO: 50 - protein, 449 aa, synthetic construct
  source 1..449: note = heavy chain of hAb01_G1_V4
EVQLVESGGGLVKPGGSLRLSCAASGFTLSDYYIYWVRQAPGKGLEWVATISDAVIYTYYADSVKGRFTISRDNAKNSLYLQMNSLRAEDTAVYFCARAYGSSEVMDYWGQGTLVTVSSASTKGPSVFPLAPSSKSTSGGTAALGCLVKDYFPEPVTVSWNSGALTSGVHTFPAVLQSSGLYSLSSVVTVPSSSLGTQTYICNVNHKPSNTKVDKKVEPKSCDKTHTCPPCPAPEAAGGPSVFLFPPKPKDTLYITREPEVTCVVVDVSHEDPEVKFNWYVDGVEVHNAKTKPREEQYNSTYRVVSVLTVLHQDWLNGKEYKCKVSNKALPAPIEKTISKAKGQPREPQVYTLPPSRDELTKNQVSLTCLVKGFYPSDIAVEWESNGQPENNYKTTPPVLDSDGSFFLYSKLTVDKSRWQQGNVFSCSVMHEALHNHYTQKSLSLSPGK

SEQ ID NO: 51 - protein, 213 aa, synthetic construct
  source 1..213: note = light chain of hAb01_G4P/hAb01_G4P_V1/hAb01_G4P_V2/hAb01_G1/hAb01_G1_V4
EIVLTQSPATLSLSPGERATLSCSASSSVSYMHWYQQKPGQAPKRWIYDTSKLASGVPARFSGSGSGTDYTLTISSLEPEDFAVYYCQQWSSNPWTFGGGTKLEIKRTVAAPSVFIFPPSDEQLKSGTASVVCLLNNFYPREAKVQWKVDNALQSGNSQESVTEQDSKDSTYSLSSTLTLSKADYEKHKVYACEVTHQGLSSPVTKSFNRGEC

SEQ ID NO: 52 - DNA, 20 bp, synthetic construct
  source 1..20: mol_type = other DNA; note = forward primer (TPO)
tgcagttggctgagaagagg

SEQ ID NO: 53 - DNA, 20 bp, synthetic construct
  source 1..20: mol_type = other DNA; note = reverse primer (TPO)
tctgtgcaggccataaccag

SEQ ID NO: 54 - DNA, 20 bp, synthetic construct
  source 1..20: mol_type = other DNA; note = forward primer (GAPDH)
atcatccctgcctctactgg

SEQ ID NO: 55 - DNA, 19 bp, synthetic construct
  source 1..19: mol_type = other DNA; note = reverse primer (GAPDH)
tgggtgcgctgttgaagtc